European Patent Specification EP 3 247 384 B1, published October 4, 2023. Title: INSULIN MIMOTOPES AND METHODS OF USING THE SAME. Applicant: The Regents of the University of Colorado, a body corporate National Jewish Health Michels, Aaron Kappler, John Gottlieb, Peter A. Application Not yet assigned. The sequence listing filed with the application follows.

SEQUENCE LISTING (27 sequences)

SEQ ID NO: 1 - protein, 15 aa, Homo sapiens
SHLVEALYLVCGERG

SEQ ID NO: 2 - protein, 15 aa, Artificial Sequence
  Synthetic Peptide
SHLVEALYLVCGEEG

SEQ ID NO: 3 - protein, 15 aa, Artificial Sequence
  Synthetic Peptide
SHLVEALYLVCGGEG

SEQ ID NO: 4 - protein, 15 aa, Artificial Sequence
  Synthetic Peptide
SHLVEELYLVCGEEG

SEQ ID NO: 5 - protein, 15 aa, Artificial Sequence
  Synthetic Peptide
SHLVEELYLVCGERG

SEQ ID NO: 6 - protein, 15 aa, Artificial Sequence
  Synthetic Peptide
SHLVGELYLVCGERG

SEQ ID NO: 7 - protein, 15 aa, Artificial Sequence
  Synthetic Peptide
SHLVGELYLVCGGEG

SEQ ID NO: 8 - protein, 15 aa, Artificial Sequence
  Synthetic Peptide
SHLVGALYLVCGGEG

SEQ ID NO: 9 - protein, 15 aa, Artificial Sequence
  Synthetic Peptide
SHLVGELYLVCGGRG

SEQ ID NO: 10 - protein, 15 aa, Artificial Sequence
  Synthetic Peptide
SHLVEALYLVAGEEG

SEQ ID NO: 11 - protein, 15 aa, Artificial Sequence
  Synthetic Peptide
SHLVEALYLVAGGEG

SEQ ID NO: 12 - protein, 15 aa, Artificial Sequence
  Synthetic Peptide
SHLVEALYLVAGAEG

SEQ ID NO: 13 - protein, 15 aa, Artificial Sequence
  Synthetic Peptide
SHLVEALYLVAGVEG

SEQ ID NO: 14 - protein, 15 aa, Artificial Sequence
  Synthetic Peptide
SHLVEALYLVAGLEG

SEQ ID NO: 15 - protein, 15 aa, Artificial Sequence
  Synthetic Peptide
SHLVEALYLVAEAEG

SEQ ID NO: 16 - protein, 15 aa, Artificial Sequence
  Synthetic Peptide
SHLVEALYLVAAEDG

SEQ ID NO: 17 - protein, 15 aa, Artificial Sequence
  Synthetic Peptide
SHLVEALYLVAQVEG

SEQ ID NO: 18 - protein, 15 aa, Artificial Sequence
  Synthetic Peptide
SHLVEALYLVAALEG

SEQ ID NO: 19 - protein, 15 aa, Artificial Sequence
  Synthetic Peptide
SHLVEALYLVEAEDG

SEQ ID NO: 20 - protein, 15 aa, Artificial Sequence
  Synthetic Peptide
SHLVEALYLVGQVEG

SEQ ID NO: 21 - protein, 15 aa, Artificial Sequence
  Synthetic Peptide
SHLVEALYLVLALEG

SEQ ID NO: 22 - DNA, 31 bp, Artificial Sequence
  Synthetic Primer
ccaggccacagcactgttgctcttgaagtcc

SEQ ID NO: 23 - DNA, 27 bp, Artificial Sequence
  Synthetic Primer
gctgaccccactgtgcacctccttccc

SEQ ID NO: 24 - DNA, 53 bp, Artificial Sequence
  Synthetic Primer
cctatcccctgtgtgccttggcagtctcagaagcagtggtatcaacgcagagt

SEQ ID NO: 25 - DNA, 30 bp, Artificial Sequence
  Synthetic Primer
ccatctcatccctgcgtgtctccgactcag

SEQ ID NO: 26 - DNA, 24 bp, Artificial Sequence
  Synthetic Primer
gctggtacacggcagggtcagggt

SEQ ID NO: 27 - DNA, 24 bp, Artificial Sequence
  Synthetic Primer
cacagcgacctcgggtgggaacac